European Patent Application EP 4 421 091 A1, published August 28, 2024. Title: HUMAN FC VARIANTS HAVING IMPROVED FCΓRIIA BINDING SELECTIVITY. Applicant: KOREA UNIVERSITY RESEARCH AND BUSINESS FOUNDATION. Application KR. The sequence listing filed with the application follows.

SEQUENCE LISTING (8 sequences)

SEQ ID NO: 1 - protein, 227 aa, synthetic construct
DKTHTCPPCPAPELLAGPSVFLFPPKPKDTLMISRTPEVTCVVVDVSHEDPEVKFNWYVDGVEVHNAKTKPREEQYNSTYRVVSVLTVLHRDWLNGKEYKCKVSNKALPAPIEKTISKAKGQPREPQVYTLPPSRDELTKNQVSLTCLVKGFYPSDIAVEWESNGQPENNYKTTPLVLDSDGSFFLYSKLTVDKSRWQQGNVFSCSVLHEALHNHYTQKSLSLSPGK

SEQ ID NO: 2 - DNA, 681 bp, synthetic construct
  source 1..681: mol_type = other DNA
gacaaaactcacacatgcccaccgtgcccagcacctgaactcctggcgggaccgtcagtcttcctcttccccccaaaacccaaggacaccctcatgatctcccggacccctgaggtcacatgcgtggtagtggacgtgagccacgaagaccctgaggtcaagttcaactggtacgtggacggcgtggaggtgcataatgccaagacaaagccgcgggaggagcagtacaacagcacgtaccgtgtggtcagcgtcctcaccgtcctgcaccgtgactggctgaatggcaaggagtacaagtgcaaggtctccaacaaagccctcccagcccccatcgagaaaaccatctccaaagccaaagggcagccccgagaaccacaggtgtacaccctgcccccatcccgggatgagctgaccaagaaccaggtcagcctgacctgcctggtcaaaggcttctatcccagcgacatcgccgtggagtgggagagcaatgggcagccggagaacaactacaagaccacacctctcgtgctggactccgacggctccttcttcctctacagcaagctcaccgtggacaagagcaggtggcagcaggggaacgtcttctcatgctccgtgctgcatgaggctctgcacaaccactacacgcagaagagcctctccctgtccccgggtaaa

SEQ ID NO: 3 - protein, 227 aa, synthetic construct
DKTHTCPPRPAPELLAGPSVFLFPPKPKDTLMISRTPEVTCVVVDVSHEDPEVKFNWYVDGVEVHNAKTKPREEQYNSTYRVVSVLTVLHRDWLNGKEYKCKVSNKALPAPIEKTISKAKGQPREPQVYTLPPSRDELTKNQVSLTCLVKGFYPSDIAVEWESNGQPENNYKTTPLVLDSDGSFFLYSKLTVDKSRWQQGNVFSCSVLHEALHNHYTQKSLSLSPGK

SEQ ID NO: 4 - DNA, 681 bp, synthetic construct
  source 1..681: mol_type = other DNA
gacaaaactcacacatgcccaccgcgcccagcacctgaactcctggcgggaccgtcagtcttcctcttccccccaaaacccaaggacaccctcatgatctcccggacccctgaggtcacatgcgtggtagtggacgtgagccacgaagaccctgaggtcaagttcaactggtacgtggacggcgtggaggtgcataatgccaagacaaagccgcgggaggagcagtacaacagcacgtaccgtgtggtcagcgtcctcaccgtcctgcaccgtgactggctgaatggcaaggagtacaagtgcaaggtctccaacaaagccctcccagcccccatcgagaaaaccatctccaaagccaaagggcagccccgagaaccacaggtgtacaccctgcccccatcccgggatgagctgaccaagaaccaggtcagcctgacctgcctggtcaaaggcttctatcccagcgacatcgccgtggagtgggagagcaatgggcagccggagaacaactacaagaccacacctctcgtgctggactccgacggctccttcttcctctacagcaagctcaccgtggacaagagcaggtggcagcaggggaacgtcttctcatgctccgtgctgcatgaggctctgcacaaccactacacgcagaagagcctctccctgtccccgggtaaa

SEQ ID NO: 5 - protein, 227 aa, synthetic construct
DKTHTCPPCPVPELLWGPSVFLLPPKPKDTLMISRTPEVTCVVVDVSHEDPEVKFNWYVDGVEVHNAKTKPREEQYNSTYRVVSVLTVLHRDWLNGKEYKCKVSNKALPAPIEKTISKAKGQPREPQVYTLPPSLDELTKNQVSLTCLVKGFYPSDIAVEWESNGQPENNYKTTPLVLDSDGSFFLYSKLTVDKSRWQQGNVFSCSVLHEALHNHYTQKSLSLSPGK

SEQ ID NO: 6 - DNA, 681 bp, synthetic construct
  source 1..681: mol_type = other DNA
gacaaaactcacacatgcccaccgtgcccagtacctgaactcctgtggggaccgtcagtcttcctcctccccccaaaacccaaggacaccctcatgatctcccggacccctgaggtcacatgcgtggtggtggacgtgagccacgaagaccctgaggtcaagttcaactggtacgtggacggcgtggaggtgcataatgccaagacaaagccgcgggaggagcagtacaacagcacgtaccgtgtggtcagcgtcctcaccgtcctgcaccgtgactggctgaatggcaaggagtacaagtgcaaggtctccaacaaagccctcccagcccccatcgagaaaaccatctccaaagccaaagggcagccccgagaaccacaggtgtacaccctgcccccatccctggatgagctgaccaagaaccaggtcagcctgacctgcctggtcaaaggcttctatcccagcgacatcgccgtggagtgggagagcaatgggcagccggagaacaactacaagaccacacctctcgtgctggactccgacggctccttcttcctctacagcaagctcaccgtggacaagagcaggtggcagcaggggaacgtcttctcatgctccgtgctgcatgaggctctgcataaccactacacgcagaagagcctctccctgtccccgggtaaa

SEQ ID NO: 7 - protein, 227 aa, synthetic construct
DKTHTCPPCPAPELLGGPSVFLFPPKPKDTLMISRTPEVTCVVVDVSHEDPEVKFNWYVDGVEVHNAKTKPREEQYNSTYRVVSVLTVLHQDWLNGKEYKCKVSNKALPAPIEKTISKAKGQPREPQVYTLPPSRDELTKNQVSLTCLVKGFYPSDIAVEWESNGQPENNYKTTPPVLDSDGSFFLYSKLTVDKSRWQQGNVFSCSVMHEALHNHYTQKSLSLSPGK

SEQ ID NO: 8 - DNA, 681 bp, synthetic construct
  source 1..681: mol_type = other DNA
gacaaaactcacacatgcccaccgtgcccagcacctgaactcctggggggaccgtcagtcttcctcttccccccaaaacccaaggacaccctcatgatctcccggacccctgaggtcacatgcgtggtggtggacgtgagccacgaagaccctgaggtcaagttcaactggtacgtggacggcgtggaggtgcataatgccaagacaaagccgcgggaggagcagtacaacagcacgtaccgtgtggtcagcgtcctcaccgtcctgcaccaggactggctgaatggcaaggagtacaagtgcaaggtctccaacaaagccctcccagcccccatcgagaaaaccatctccaaagccaaagggcagccccgagaaccacaggtgtacaccctgcccccatcccgggatgagctgaccaagaaccaggtcagcctgacctgcctggtcaaaggcttctatcccagcgacatcgccgtggagtgggagagcaatgggcagccggagaacaactacaagaccacacctcccgtgctggactccgacggctccttcttcctctacagcaagctcaccgtggacaagagcaggtggcagcaggggaacgtcttctcatgctccgtgatgcatgaggctctgcacaaccactacacgcagaagagcctctccctgtccccgggtaaa